European Patent Application EP 4 361 168 A1, published May 1, 2024. Title: INSECT NEUROPEPTIDES 6. Applicant: SOLASTA Bio Limited. The sequence listing filed with the application follows.

SEQUENCE LISTING (16 sequences)

SEQ ID NO: 1 - protein, 10 aa, synthetic construct
  source 1..10: note = Z peptide
RQKTVFSSWG

SEQ ID NO: 2 - protein, 10 aa, synthetic construct
  source 1..10: note = SB-P-65
  MOD_RES 10: note = glycinamide
RQKTVFSSWG

SEQ ID NO: 3 - protein, 11 aa, synthetic construct
  source 1..11: note = SB-P-47
  MOD_RES 11: note = leucinamide
  MOD_RES 1: note = pyroglutamyl-alanine
AIMARPQVPRL

SEQ ID NO: 4 - protein, 8 aa, synthetic construct
  source 1..8: note = SB-P-49
  MOD_RES 8: note = leucinamide
SVPFKPRL

SEQ ID NO: 5 - protein, 19 aa, synthetic construct
  source 1..19: note = SB-P-51
  MOD_RES 19: note = leucinamide
LRQLQSNGEPAYRVRTPRL

SEQ ID NO: 6 - protein, 16 aa, synthetic construct
  source 1..16: note = SB-P-80
  MOD_RES 16: note = leucinamide
NADEDQQQSVDFTPRL

SEQ ID NO: 7 - protein, 10 aa, synthetic construct
  source 1..10: note = SB-P-81
  MOD_RES 10: note = leucinamide
GGSMTFSPRL

SEQ ID NO: 8 - protein, 8 aa, synthetic construct
  source 1..8: note = SB-P-70
  MOD_RES 8: note = glycinamide
KVKFSAWG

SEQ ID NO: 9 - protein, 12 aa, synthetic construct
  source 1..12: note = SB-P-46
  MOD_RES 12: note = leucinamide
SPPYSPPFSPRL

SEQ ID NO: 10 - protein, 7 aa, synthetic construct
  source 1..7: note = SB-P-66
  MOD_RES 7: note = glycinamide
PAFSSWG

SEQ ID NO: 11 - protein, 9 aa, synthetic construct
  source 1..9: note = SB-P-86
  MOD_RES 9: note = glycinamide
  MOD_RES 1: note = pyroglutamyl-leucine
LTFTSSWGG

SEQ ID NO: 12 - protein, 8 aa, synthetic construct
  source 1..8: note = SB-P-039
  MOD_RES 1: note = palmitoyl-glutamine
  MOD_RES 8: note = tryptophanamide
QLTFSPDW

SEQ ID NO: 13 - protein, 7 aa, synthetic construct
  source 1..7: note = SB-P-042
  MOD_RES 1: note = pyroglutamyl-leucine
  MOD_RES 7: note = tryptophanamide
LTFSPDW

SEQ ID NO: 14 - protein, 6 aa, synthetic construct
  source 1..6: note = SB-P-69
  MOD_RES 6: note = glycinamide
NFSPWG

SEQ ID NO: 15 - protein, 19 aa, synthetic construct
  source 1..19: note = SB-P-48
  MOD_RES 19: note = leucinamide
EQNVQSNGEPAYRVRTPRL

SEQ ID NO: 16 - protein, 8 aa, synthetic construct
  source 1..8: note = SB-P-41
  MOD_RES 8: note = tryptophanamide
QLTFSPDW